European Patent Application EP 4 249 912 A1, published September 27, 2023. Title: Phosphorylation of P53 as a prognostic or diagnostic marker for the treatment of senescent cells in a mammal. Applicant: Cleara Biotech B.V. The sequence listing filed with the application follows.

SEQUENCE LISTING (9 sequences)

SEQ ID NO: 1 - protein, 37 aa, Homo Sapiens
RKKASSKIEAAILDAFSQNWRFFKRPPRRRQRRKKRG

SEQ ID NO: 2 - protein, 36 aa, Homo Sapiens
RKKASSKIEAEILDAFSQNWRRKRPPRRRQRRKKRG

SEQ ID NO: 3 - protein, 28 aa, Homo Sapiens
AKIEAAILDAFSQNWRKRRRRQRRKKRG

SEQ ID NO: 4 - protein, 17 aa, Homo Sapiens
KIEAEILDAFSQNWRKR

SEQ ID NO: 5 - protein, 17 aa, Homo Sapiens
KIEAAILDAFSQNWRKR

SEQ ID NO: 6 - protein, 17 aa, Homo Sapiens
KIEAAILDAFSQNWRKR

SEQ ID NO: 7 - protein, 34 aa, Homo Sapiens
LTLRKEPASEIAQSILEAYSQNGWANRRSGGKRP

SEQ ID NO: 8 - protein, 12 aa, Human immunodeficiency virus
GRKKRRQRRRPP

SEQ ID NO: 9 - protein, 13 aa, TAT sequence
ARKKRRQRRRPPP